European Patent Specification EP 4 504 933 B1, published June 3, 2026. Title: Method. Applicant: OXFORD NANOPORE TECHNOLOGIES PLC. The sequence listing filed with the application follows.

SEQUENCE LISTING (78 sequences)

SEQ ID NO: 1 - DNA, 91 bp, synthetic construct
  source 1..91: mol_type = other DNA
  misc_feature 1: note = click group to facilitate downstream attachment to sequencing adapter (DBCO-TEG) dT tail
gcttgggtgtttaaccaaaaggttacacaaaccctggacaagccatatccgtgtcgcccttattccgatagtgactacagcggcatgagtg

SEQ ID NO: 2 - DNA, 49 bp, synthetic construct
  source 1..49: mol_type = other DNA
  modified_base 45: mod_base = um
  modified_base 46: mod_base = um
  modified_base 47: mod_base = um
  modified_base 48: mod_base = um
  modified_base 49: mod_base = um
  misc_feature 1: note = 5Phos dT tail
agggcgacacggatatggcttgtccagggtttgtgtaaccttttnnnnn

SEQ ID NO: 3 - DNA, 18 bp, synthetic construct
  source 1..18: mol_type = other DNA
  misc_feature 1: note = 5Phos dT tail
tgtagtcactatcggaat

SEQ ID NO: 4 - DNA, 91 bp, synthetic construct; identical to SEQ ID NO: 1
  source 1..91: mol_type = other DNA
  misc_feature 1: note = click group to facilitate downstream attachment to sequencing adapter (DBCO-TEG) blunt

SEQ ID NO: 5 - DNA, 50 bp, synthetic construct
  misc_feature 1: note = 5Phos blunt
  source 1..50: mol_type = other DNA
  modified_base 45: mod_base = um
  modified_base 46: mod_base = um
  modified_base 47: mod_base = um
  modified_base 48: mod_base = um
  modified_base 49: mod_base = um
aagggcgacacggatatggcttgtccagggtttgtgtaaccttttnnnnn

SEQ ID NO: 6 - DNA, 18 bp, synthetic construct
  source 1..18: mol_type = other DNA
  misc_feature 1: note = 5Phos blunt
tgtagtcactatcggaat

SEQ ID NO: 7 - DNA, 19 bp, synthetic construct
  source 1..19: mol_type = other DNA
cttttgcacgcaattgcgc

SEQ ID NO: 8 - DNA, 19 bp, synthetic construct
  source 1..19: mol_type = other DNA
agcagtcctgtcatgtgcg

SEQ ID NO: 9 - DNA, 19 bp, synthetic construct
  source 1..19: mol_type = other DNA
tgacagacacgacgttgcc

SEQ ID NO: 10 - DNA, 19 bp, synthetic construct
  source 1..19: mol_type = other DNA
cgatcgctagcatgttggc

SEQ ID NO: 11 - DNA, 20 bp, synthetic construct
  source 1..20: mol_type = other DNA
tcatcatcaacgggaccgag

SEQ ID NO: 12 - DNA, 20 bp, synthetic construct
  source 1..20: mol_type = other DNA
acacgatctcgtcgctaacc

SEQ ID NO: 13 - DNA, 22 bp, synthetic construct
  source 1..22: mol_type = other DNA
nnncttttgcacgcaattgcgc

SEQ ID NO: 14 - DNA, 22 bp, synthetic construct
  source 1..22: mol_type = other DNA
nnnagcagtcctgtcatgtgcg

SEQ ID NO: 15 - DNA, 22 bp, synthetic construct
  source 1..22: mol_type = other DNA
nnntgacagacacgacgttgcc

SEQ ID NO: 16 - DNA, 22 bp, synthetic construct
  source 1..22: mol_type = other DNA
nnncgatcgctagcatgttggc

SEQ ID NO: 17 - DNA, 23 bp, synthetic construct
  source 1..23: mol_type = other DNA
nnntcatcatcaacgggaccgag

SEQ ID NO: 18 - DNA, 23 bp, synthetic construct
  source 1..23: mol_type = other DNA
nnnacacgatctcgtcgctaacc

SEQ ID NO: 19 - DNA, 22 bp, synthetic construct
  source 1..22: mol_type = other DNA
ggkcttttgcacgcaattgcgc

SEQ ID NO: 20 - DNA, 22 bp, synthetic construct
  source 1..22: mol_type = other DNA
ggkagcagtcctgtcatgtgcg

SEQ ID NO: 21 - DNA, 22 bp, synthetic construct
  source 1..22: mol_type = other DNA
ggktgacagacacgacgttgcc

SEQ ID NO: 22 - DNA, 22 bp, synthetic construct
  source 1..22: mol_type = other DNA
ggkcgatcgctagcatgttggc

SEQ ID NO: 23 - DNA, 23 bp, synthetic construct
  source 1..23: mol_type = other DNA
ggktcatcatcaacgggaccgag

SEQ ID NO: 24 - DNA, 23 bp, synthetic construct
  source 1..23: mol_type = other DNA
ggkacacgatctcgtcgctaacc

SEQ ID NO: 25 - DNA, 20 bp, synthetic construct
  source 1..20: mol_type = other DNA
cgaaggcatgagtttctccg

SEQ ID NO: 26 - DNA, 20 bp, synthetic construct
  source 1..20: mol_type = other DNA
cgaaggcatgagtttctccg

SEQ ID NO: 27 - DNA, 20 bp, synthetic construct
  source 1..20: mol_type = other DNA
gacgagatcctgaaacgtgc

SEQ ID NO: 28 - DNA, 20 bp, synthetic construct
  source 1..20: mol_type = other DNA
gacgagatcctgaaacgtgc

SEQ ID NO: 29 - DNA, 20 bp, synthetic construct
  source 1..20: mol_type = other DNA
gtgctggaaatcgtgcgtat

SEQ ID NO: 30 - DNA, 20 bp, synthetic construct
  source 1..20: mol_type = other DNA
gtgctggaaatcgtgcgtat

SEQ ID NO: 31 - DNA, 20 bp, synthetic construct
  source 1..20: mol_type = other DNA
cccataagacgtcagcaagc

SEQ ID NO: 32 - DNA, 20 bp, synthetic construct
  source 1..20: mol_type = other DNA
cccataagacgtcagcaagc

SEQ ID NO: 33 - DNA, 20 bp, synthetic construct
  source 1..20: mol_type = other DNA
caacatcatcctcgcaccag

SEQ ID NO: 34 - DNA, 20 bp, synthetic construct
  source 1..20: mol_type = other DNA
caacatcatcctcgcaccag

SEQ ID NO: 35 - DNA, 20 bp, synthetic construct
  source 1..20: mol_type = other DNA
ttacggttcatcagcatgcg

SEQ ID NO: 36 - DNA, 20 bp, synthetic construct
  source 1..20: mol_type = other DNA
ttacggttcatcagcatgcg

SEQ ID NO: 37 - DNA, 20 bp, synthetic construct
  source 1..20: mol_type = other DNA
cactgcctggccgtaaatac

SEQ ID NO: 38 - DNA, 20 bp, synthetic construct
  source 1..20: mol_type = other DNA
cactgcctggccgtaaatac

SEQ ID NO: 39 - DNA, 20 bp, synthetic construct
  source 1..20: mol_type = other DNA
cgtggattaagcaggtgagc

SEQ ID NO: 40 - DNA, 20 bp, synthetic construct
  source 1..20: mol_type = other DNA
cgtggattaagcaggtgagc

SEQ ID NO: 41 - DNA, 20 bp, synthetic construct
  source 1..20: mol_type = other DNA
ttccctgctgctcaatacca

SEQ ID NO: 42 - DNA, 20 bp, synthetic construct
  source 1..20: mol_type = other DNA
ttccctgctgctcaatacca

SEQ ID NO: 43 - DNA, 20 bp, synthetic construct
  source 1..20: mol_type = other DNA
cgaatccgcctgcaacataa

SEQ ID NO: 44 - DNA, 20 bp, synthetic construct
  source 1..20: mol_type = other DNA
cgaatccgcctgcaacataa

SEQ ID NO: 45 - DNA, 20 bp, synthetic construct
  source 1..20: mol_type = other DNA
gtgaatacttcctgccgcag

SEQ ID NO: 46 - DNA, 20 bp, synthetic construct
  source 1..20: mol_type = other DNA
gtgaatacttcctgccgcag

SEQ ID NO: 47 - DNA, 20 bp, synthetic construct
  source 1..20: mol_type = other DNA
gccgtaatgttaagcgcaga

SEQ ID NO: 48 - DNA, 20 bp, synthetic construct
  source 1..20: mol_type = other DNA
gccgtaatgttaagcgcaga

SEQ ID NO: 49 - DNA, 23 bp, synthetic construct
  source 1..23: mol_type = other DNA
ggkcgaaggcatgagtttctccg

SEQ ID NO: 50 - DNA, 23 bp, synthetic construct
  source 1..23: mol_type = other DNA
ggktgtcgtaatgaatgctgccg

SEQ ID NO: 51 - DNA, 23 bp, synthetic construct
  source 1..23: mol_type = other DNA
ggkgacgagatcctgaaacgtgc

SEQ ID NO: 52 - DNA, 23 bp, synthetic construct
  source 1..23: mol_type = other DNA
ggktcaggtatttgctgcccaga

SEQ ID NO: 53 - DNA, 23 bp, synthetic construct
  source 1..23: mol_type = other DNA
ggkgtgctggaaatcgtgcgtat

SEQ ID NO: 54 - DNA, 23 bp, synthetic construct
  source 1..23: mol_type = other DNA
ggkacgcgttctttatcgccttc

SEQ ID NO: 55 - DNA, 23 bp, synthetic construct
  source 1..23: mol_type = other DNA
ggkcccataagacgtcagcaagc

SEQ ID NO: 56 - DNA, 23 bp, synthetic construct
  source 1..23: mol_type = other DNA
ggkggtcataaaacggcgctgat

SEQ ID NO: 57 - DNA, 23 bp, synthetic construct
  source 1..23: mol_type = other DNA
ggkcaacatcatcctcgcaccag

SEQ ID NO: 58 - DNA, 23 bp, synthetic construct
  source 1..23: mol_type = other DNA
ggkcaaagaatcgccggaagagg

SEQ ID NO: 59 - DNA, 23 bp, synthetic construct
  source 1..23: mol_type = other DNA
ggkttacggttcatcagcatgcg

SEQ ID NO: 60 - DNA, 23 bp, synthetic construct
  source 1..23: mol_type = other DNA
ggkagatggggcagaaaatggga

SEQ ID NO: 61 - DNA, 23 bp, synthetic construct
  source 1..23: mol_type = other DNA
ggkcactgcctggccgtaaatac

SEQ ID NO: 62 - DNA, 23 bp, synthetic construct
  source 1..23: mol_type = other DNA
ggkgttgatgcgctcggtaatgt

SEQ ID NO: 63 - DNA, 23 bp, synthetic construct
  source 1..23: mol_type = other DNA
ggkcgtggattaagcaggtgagc

SEQ ID NO: 64 - DNA, 23 bp, synthetic construct
  source 1..23: mol_type = other DNA
ggkgatcacatgcagcacacgat

SEQ ID NO: 65 - DNA, 23 bp, synthetic construct
  source 1..23: mol_type = other DNA
ggkttccctgctgctcaatacca

SEQ ID NO: 66 - DNA, 23 bp, synthetic construct
  source 1..23: mol_type = other DNA
ggkttggtccgattactgggctt

SEQ ID NO: 67 - DNA, 23 bp, synthetic construct
  source 1..23: mol_type = other DNA
ggkcgaatccgcctgcaacataa

SEQ ID NO: 68 - DNA, 23 bp, synthetic construct
  source 1..23: mol_type = other DNA
ggkgcagaaatccgcgaacagat

SEQ ID NO: 69 - DNA, 23 bp, synthetic construct
  source 1..23: mol_type = other DNA
ggkgtgaatacttcctgccgcag

SEQ ID NO: 70 - DNA, 23 bp, synthetic construct
  source 1..23: mol_type = other DNA
ggkccagttgatgatggtgagcg

SEQ ID NO: 71 - DNA, 23 bp, synthetic construct
  source 1..23: mol_type = other DNA
ggkgccgtaatgttaagcgcaga

SEQ ID NO: 72 - DNA, 23 bp, synthetic construct
  source 1..23: mol_type = other DNA
ggktggatgaactgcaggatggt

SEQ ID NO: 73 - DNA, 20 bp, synthetic construct
  source 1..20: mol_type = other DNA
cgaaggcatgagtttctccg

SEQ ID NO: 74 - DNA, 20 bp, synthetic construct
  source 1..20: mol_type = other DNA
cgaaggcatgagtttctccg

SEQ ID NO: 75 - DNA, 23 bp, synthetic construct
  source 1..23: mol_type = other DNA
ggkcgaaggcatgagtttctccg

SEQ ID NO: 76 - DNA, 23 bp, synthetic construct
  source 1..23: mol_type = other DNA
ggktgtcgtaatgaatgctgccg

SEQ ID NO: 77 - DNA, 23 bp, synthetic construct
  source 1..23: mol_type = other DNA
acacgaaggcatgagtttctccg

SEQ ID NO: 78 - DNA, 23 bp, synthetic construct
  source 1..23: mol_type = other DNA
acatgtcgtaatgaatgctgccg